European Patent Specification EP 3 068 217 B1, published January 4, 2023. Title: Recombination activating gene 2 gene targeting vector, production of SCID-like miniature pigs by TALEN-mediated gene targeting and use thereof. Applicant: Konkuk University Industrial Cooperation Corp. The sequence listing filed with the application follows.

SEQUENCE LISTING (19 sequences)

SEQ ID NO: 1 - DNA, 52 bp, Sus scrofa
ttcctgaaggcagatatggtcattccattgatgtcgtgtatagtcgagggaa

SEQ ID NO: 2 - DNA, 20 bp, Artificial Sequence
  primer
gctggctaagaaggcgatta

SEQ ID NO: 3 - DNA, 21 bp, Artificial Sequence
  primer
tccccttctggaggttagaaa

SEQ ID NO: 4 - DNA, 24 bp, Artificial Sequence
  primer
aaggattcctgctaccttcctcct

SEQ ID NO: 5 - DNA, 24 bp, Artificial Sequence
  primer
agatagcccatcttgaagttctgg

SEQ ID NO: 6 - DNA, 20 bp, Artificial Sequence
  primer
tgccacatgatgcctttcta

SEQ ID NO: 7 - DNA, 20 bp, Artificial Sequence
  primer
tgctggttcaagatgctgtc

SEQ ID NO: 8 - DNA, 20 bp, Artificial Sequence
  primer
cctaggcctgagtgtgggta

SEQ ID NO: 9 - DNA, 20 bp, Artificial Sequence
  primer
gccctgacgcttttattctg

SEQ ID NO: 10 - DNA, 20 bp, Artificial Sequence
  primer
tccttgcttcccttgactgt

SEQ ID NO: 11 - DNA, 20 bp, Artificial Sequence
  primer
cgagagcatttctcgtagcc

SEQ ID NO: 12 - DNA, 20 bp, Artificial Sequence
  primer
tgtgcagttttcaaccatcc

SEQ ID NO: 13 - DNA, 20 bp, Artificial Sequence
  primer
gtctttcagtccccctttcc

SEQ ID NO: 14 - DNA, 20 bp, Artificial Sequence
  primer
acaagtggcctttcatgacc

SEQ ID NO: 15 - DNA, 20 bp, Artificial Sequence
  primer
ctcttcctccagctcctcct

SEQ ID NO: 16 - DNA, 23 bp, Artificial Sequence
  primer
cactaaatagtggccttcttgga

SEQ ID NO: 17 - DNA, 20 bp, Artificial Sequence
  primer
acacacccatccttttccag

SEQ ID NO: 18 - DNA, 21 bp, Artificial Sequence
  primer
gaaatgggtttgttgagtcca

SEQ ID NO: 19 - DNA, 20 bp, Artificial Sequence
  primer
acggtggcagagctgaatag